European Patent Application EP 4 309 676 A1, published January 24, 2024. Title: Novel Anti-Nectin-4-Antibody Camptothecin derivative Conjugates. Applicant: Emergence Therapeutics AG et al. The sequence listing filed with the application follows.

SEQUENCE LISTING (125 sequences)

SEQ ID NO: 1 - protein, 8 aa, synthetic construct
  REGION 1..8: note = CDR1 VH_15A7.5 IMGT
GFTFSNYG

SEQ ID NO: 2 - protein, 8 aa, synthetic construct
  REGION 1..8: note = CDR2 VH_15A7.5 IMGT
ISNLAYGI

SEQ ID NO: 3 - protein, 12 aa, synthetic construct
  REGION 1..12: note = CDR3 VH_15A7.5 IMGT
ARGARATGWFAY

SEQ ID NO: 4 - protein, 6 aa, synthetic construct
  REGION 1..6: note = CDR1 VK_15A7.5 IMGT
QNVDTH

SEQ ID NO: 5 - skipped

SEQ ID NO: 6 - protein, 9 aa, synthetic construct
  REGION 1..9: note = CDR3 VK_15A7.5 IMGT
QQYNSYPLT

SEQ ID NO: 7 - protein, 5 aa, synthetic construct
  REGION 1..5: note = CDR1 VH_15A7.5 Kabat
NYGMA

SEQ ID NO: 8 - protein, 17 aa, synthetic construct
  REGION 1..17: note = CDR2 VH_15A7.5 Kabat
FISNLAYGINYADTVTG

SEQ ID NO: 9 - protein, 10 aa, synthetic construct
  REGION 1..10: note = CDR3 VH_15A7.5 Kabat
GARATGWFAY

SEQ ID NO: 10 - protein, 11 aa, synthetic construct
  REGION 1..11: note = CDR1 VK_15A7.5 Kabat
KASQNVDTHVA

SEQ ID NO: 11 - protein, 7 aa, synthetic construct
  REGION 1..7: note = CDR2 VK_15A7.5 Kabat
SASYRYS

SEQ ID NO: 12 - protein, 9 aa, synthetic construct
  REGION 1..9: note = CDR3 VK_15A7.5 Kabat
QQYNSYPLT

SEQ ID NO: 13 - protein, 119 aa, synthetic construct
  REGION 1..119: note = VH_15A7.5
EVKLVESGGGLVQPGGSRKLSCAASGFTFSNYGMAWVRQAPGKGPEWVAFISNLAYGINYADTVTGRFTISRENAKNTLYLEMRSLRSEDTAMYYCARGARATGWFAYWGQGTLVTVSA

SEQ ID NO: 14 - protein, 107 aa, synthetic construct
  REGION 1..107: note = VK_15A7.5
DIVMTQSQKFMSTSIGDRVSVTCKASQNVDTHVAWYQEKPGQSPKALIYSASYRYSGVPDRFTGSGSGTDFTLTISNVQSEDLADYFCQQYNSYPLTFGGGTKLEIK

SEQ ID NO: 15 - protein, 9 aa, synthetic construct
  REGION 1..9: note = CDR1 H0_15A7.5IMGT
GFTFSNYGM

SEQ ID NO: 16 - protein, 8 aa, synthetic construct
  REGION 1..8: note = CDR2 H0_15A7.5IMGT
ISNLAYGI

SEQ ID NO: 17 - protein, 12 aa, synthetic construct
  REGION 1..12: note = CDR3 H0_15A7.5IMGT
ARGARATGWFAY

SEQ ID NO: 18 - protein, 6 aa, synthetic construct
  REGION 1..6: note = CDR1 L0_15A7.5 IMGT
QNVDTH

SEQ ID NO: 19 - skipped

SEQ ID NO: 20 - protein, 9 aa, synthetic construct
  REGION 1..9: note = CDR3 L0_15A7.5 IMGT
QQYNSYPLT

SEQ ID NO: 21 - protein, 5 aa, synthetic construct
  REGION 1..5: note = CDR1 H0_15A7.5Kabat
NYGMN

SEQ ID NO: 22 - protein, 17 aa, synthetic construct
  REGION 1..17: note = CDR2 H0_15A7.5Kabat
FISNLAYGINYADSVKG

SEQ ID NO: 23 - protein, 10 aa, synthetic construct
  REGION 1..10: note = CDR3 H0_15A7.5Kabat
GARATGWFAY

SEQ ID NO: 24 - protein, 11 aa, synthetic construct
  REGION 1..11: note = CDR1 L0_15A7.5 Kabat
RASQNVDTHVA

SEQ ID NO: 25 - protein, 7 aa, synthetic construct
  REGION 1..7: note = CDR2 L0_15A7.5 Kabat
SASYLQS

SEQ ID NO: 26 - protein, 9 aa, synthetic construct
  REGION 1..9: note = CDR3 L0_15A7.5 Kabat
QQYNSYPLT

SEQ ID NO: 27 - protein, 119 aa, synthetic construct
  REGION 1..119: note = H0_15A7.5
EVQLVESGGGLVQPGGSLRLSCAASGFTFSNYGMNWVRQAPGKGLEWVSFISNLAYGINYADSVKGRFTISRDNAKNSLYLQMNSLRAEDTAVYYCARGARATGWFAYWGQGTLVTVSS

SEQ ID NO: 28 - protein, 107 aa, synthetic construct
  REGION 1..107: note = L0_15A7.5
DIQMTQSPSSLSASVGDRVTITCRASQNVDTHVAWFQQKPGKAPKSLIYSASYLQSGVPSRFSGSGSGTDFTLTISSLQPEDFATYYCQQYNSYPLTFGGGTKVEIK

SEQ ID NO: 29 - protein, 8 aa, synthetic construct
  REGION 1..8: note = CDR1 H1_15A7.5 IMGT
GFTFSNYG

SEQ ID NO: 30 - protein, 8 aa, synthetic construct
  REGION 1..8: note = CDR2 H1_15A7.5 IMGT
ISNLAYGI

SEQ ID NO: 31 - protein, 12 aa, synthetic construct
  REGION 1..12: note = CDR3 H1_15A7.5 IMGT
ARGARATGWFAY

SEQ ID NO: 32 - protein, 6 aa, synthetic construct
  REGION 1..6: note = CDR1 L1_15A7.5 IMGT
QNVDTH

SEQ ID NO: 33 - skipped

SEQ ID NO: 34 - protein, 9 aa, synthetic construct
  REGION 1..9: note = CDR3 L1_15A7.5 IMGT
QQYNSYPLT

SEQ ID NO: 35 - protein, 5 aa, synthetic construct
  REGION 1..5: note = CDR1 H1_15A7.5 Kabat
NYGMA

SEQ ID NO: 36 - protein, 17 aa, synthetic construct
  REGION 1..17: note = CDR2 H1_15A7.5 Kabat
FISNLAYGINYADTVTG

SEQ ID NO: 37 - protein, 10 aa, synthetic construct
  REGION 1..10: note = CDR3 H1_15A7.5 Kabat
GARATGWFAY

SEQ ID NO: 38 - protein, 11 aa, synthetic construct
  REGION 1..11: note = CDR1 L1_15A7.5 Kabat
KASQNVDTHVA

SEQ ID NO: 39 - protein, 7 aa, synthetic construct
  REGION 1..7: note = CDR2 L1_15A7.5 Kabat
SASYRYS

SEQ ID NO: 40 - protein, 9 aa, synthetic construct
  REGION 1..9: note = CDR3 L1_15A7.5 Kabat
QQYNSYPLT

SEQ ID NO: 41 - protein, 119 aa, synthetic construct
  REGION 1..119: note = H1_15A7.5
EVQLVESGGGLVQPGGSLRLSCAASGFTFSNYGMAWVRQAPGKGLEWVSFISNLAYGINYADTVTGRFTISRDNAKNSLYLQMNSLRAEDTAVYYCARGARATGWFAYWGQGTLVTVSS

SEQ ID NO: 42 - protein, 108 aa, synthetic construct
  REGION 1..108: note = L1_15A7.5
DIQMTQSPSSLSASVGDRVTITCCKASQNVDTHVAWFQQKPGKAPKSLIYSASYRYSGVPSRFSGSGSGTDFTLTISSLQPEDFATYYCQQYNSYPLTFGGGTKVEIK

SEQ ID NO: 43 - protein, 8 aa, synthetic construct
  REGION 1..8: note = CDR1 H2_15A7.5 IMGT
GFTFSNYG

SEQ ID NO: 44 - protein, 8 aa, synthetic construct
  REGION 1..8: note = CDR2 H2_15A7.5 IMGT
ISNLAYGI

SEQ ID NO: 45 - protein, 12 aa, synthetic construct
  REGION 1..12: note = CDR3 H2_15A7.5 IMGT
ARGARATGWFAY

SEQ ID NO: 46 - protein, 6 aa, synthetic construct
  REGION 1..6: note = CDR1 L2_15A7.5 IMGT
QNVDTH

SEQ ID NO: 47 - skipped

SEQ ID NO: 48 - protein, 9 aa, synthetic construct
  REGION 1..9: note = CDR3 L2_15A7.5 IMGT
QQYNSYPLT

SEQ ID NO: 49 - protein, 5 aa, synthetic construct
  REGION 1..5: note = CDR1 H2_15A7.5 Kabat
NYGMA

SEQ ID NO: 50 - protein, 17 aa, synthetic construct
  REGION 1..17: note = CDR2 H2_15A7.5 Kabat
FISNLAYGINYADTVTG

SEQ ID NO: 51 - protein, 10 aa, synthetic construct
  REGION 1..10: note = CDR3 H2_15A7.5 Kabat
GARATGWFAY

SEQ ID NO: 52 - protein, 11 aa, synthetic construct
  REGION 1..11: note = CDR1 L2_15A7.5 Kabat
KASQNVDTHVA

SEQ ID NO: 53 - protein, 7 aa, synthetic construct
  REGION 1..7: note = CDR2 L2_15A7.5 Kabat
SASYRYS

SEQ ID NO: 54 - protein, 9 aa, synthetic construct
  REGION 1..9: note = CDR3 L2_15A7.5 Kabat
QQYNSYPLT

SEQ ID NO: 55 - protein, 119 aa, synthetic construct
  REGION 1..119: note = H2_15A7.5
EVQLVESGGGLVQPGGSLRLSCAASGFTFSNYGMAWVRQAPGKGLEWVAFISNLAYGINYADTVTGRFTISRDNAKNSLYLQMNSLRAEDTAVYYCARGARATGWFAYWGQGTLVTVSS

SEQ ID NO: 56 - protein, 107 aa, synthetic construct
  REGION 1..107: note = L2_15A7.5
DIQMTQSPSSLSASVGDRVTITCKASQNVDTHVAWYQQKPGKAPKALIYSASYRYSGVPSRFSGSGSGTDFTLTISSLQPEDFATYYCQQYNSYPLTFGGGTKVEIK

SEQ ID NO: 57 - protein, 8 aa, synthetic construct
  REGION 1..8: note = CDR1 H3_15A7.5 IMGT
GFTFSNYG

SEQ ID NO: 58 - protein, 8 aa, synthetic construct
  REGION 1..8: note = CDR2 H3_15A7.5 IMGT
ISNLAYGI

SEQ ID NO: 59 - protein, 12 aa, synthetic construct
  REGION 1..12: note = CDR3 H3_15A7.5 IMGT
ARGARATGWFAY

SEQ ID NO: 60 - protein, 6 aa, synthetic construct
  REGION 1..6: note = CDR1 L3_15A7.5 IMGT
QNVDTH

SEQ ID NO: 61 - skipped

SEQ ID NO: 62 - protein, 9 aa, synthetic construct
  REGION 1..9: note = CDR3 L3_15A7.5 IMGT
QQYNSYPLT

SEQ ID NO: 63 - protein, 5 aa, synthetic construct
  REGION 1..5: note = CDR1 H3_15A7.5 Kabat
NYGMA

SEQ ID NO: 64 - protein, 17 aa, synthetic construct
  REGION 1..17: note = CDR2 H3_15A7.5 Kabat
FISNLAYGINYADTVTG

SEQ ID NO: 65 - protein, 10 aa, synthetic construct
  REGION 1..10: note = CDR3 H3_15A7.5 Kabat
GARATGWFAY

SEQ ID NO: 66 - protein, 11 aa, synthetic construct
  REGION 1..11: note = CDR1 L3_15A7.5 Kabat
KASQNVDTHVA

SEQ ID NO: 67 - protein, 7 aa, synthetic construct
  REGION 1..7: note = CDR2 L3_15A7.5 Kabat
SASYRYS

SEQ ID NO: 68 - protein, 9 aa, synthetic construct
  REGION 1..9: note = CDR3 L3_15A7.5 Kabat
QQYNSYPLT

SEQ ID NO: 69 - protein, 119 aa, synthetic construct
  REGION 1..119: note = H3_15A7.5
EVQLVESGGGLVQPGGSLRLSCAASGFTFSNYGMAWVRQAPGKGPEWVAFISNLAYGINYADTVTGRFTISRDNAKNSLYLQMNSLRAEDTAVYYCARGARATGWFAYWGQGTLVTVSS

SEQ ID NO: 70 - protein, 108 aa, synthetic construct
  REGION 1..108: note = L3_15A7.5
DIQMTQSPSSLSASVGDRVTITCKASQNVDTHVAWYYQQKPGKSPKALIYSASYRYSGVPSRFSGSGSGTDFTLTISSLQPEDFATYYCQQYNSYPLTFGGGTKVEIK

SEQ ID NO: 71 - protein, 107 aa, synthetic construct
  REGION 1..107: note = L3_15A7.5_mod
DIQMTQSPSSLSASVGDRVTITCKASQNVDTHVAWYYQQKPGKSPKALIYSASYRYSGVPSRFSGSGSGTDFTLTISSLQPEDFATYCQQYNSYPLTFGGGTKVEIK

SEQ ID NO: 72 - protein, 8 aa, synthetic construct
  REGION 1..8: note = CDR1 VH_HA22
GFTFSSYN

SEQ ID NO: 73 - protein, 8 aa, synthetic construct
  REGION 1..8: note = CDR2 VH_HA22
ISSSSSTI

SEQ ID NO: 74 - protein, 10 aa, synthetic construct
  REGION 1..10: note = CDR3 VH_HA22
ARAYYYGMDV

SEQ ID NO: 75 - protein, 6 aa, synthetic construct
  REGION 1..6: note = CDR1 VK_HA22
QGISGW

SEQ ID NO: 76 - skipped

SEQ ID NO: 77 - protein, 9 aa, synthetic construct
  REGION 1..9: note = CDR3 VK_HA22
QQANSFPPT

SEQ ID NO: 78 - protein, 117 aa, synthetic construct
  REGION 1..117: note = VH_HA22
EVQLVESGGGLVQPGGSLRLSCAASGFTFSSYNMNWVRQAPGKGLEWVSYISSSSSTIYYADSVKGRFTISRDNAKNSLSLQMNSLRDEDTAVYYCARAYYYGMDVWGQGTTVTVSS

SEQ ID NO: 79 - protein, 107 aa, synthetic construct
  REGION 1..107: note = VK_HA22
DIQMTQSPSSVSASVGDRVTITCRASQGISGWLAWYQQKPGKAPKFLIYAASTLQSGVPSRFSGSGSGTDFTLTISSLQPEDFATYYCQQANSFPPTFGGGTKVEIK

SEQ ID NO: 80 - protein, 8 aa, synthetic construct
  REGION 1..8: note = CDR1 VH_5A12.2
GFTFNSMY

SEQ ID NO: 81 - protein, 8 aa, synthetic construct
  REGION 1..8: note = CDR2 VH_5A12.2
IYAGTGGT

SEQ ID NO: 82 - protein, 13 aa, synthetic construct
  REGION 1..13: note = CDR3 VH_5A12.2
AIRSGFVPMDYWG

SEQ ID NO: 83 - protein, 118 aa, synthetic construct
  REGION 1..118: note = VH_5A12.2
QIQLQQSGAELVKPGASVTLSCKTSGFTFNSMYISWLKQKPGQSLEWIAWIYAGTGGTRFNQKFTGKVQLTVDTSSSTAYMQFSSLTTDDSAIYYCAIRSGFVPMDYWGQGTSVTVSS

SEQ ID NO: 84 - protein, 6 aa, synthetic construct
  REGION 1..6: note = CDR1 VK_5A12.2
QSVSND

SEQ ID NO: 85 - skipped

SEQ ID NO: 86 - protein, 6 aa, synthetic construct
  REGION 1..6: note = CDR3 VK_5A12.2
QQDYSS

SEQ ID NO: 87 - protein, 107 aa, synthetic construct
  REGION 1..107: note = VK_5A12.2
SIVMTQTPKFLLVSAGDRVTITCKASQSVSNDVAWYQQKPGQSPKLLIYYASNRYTGVPDRFTGSGYGTDFTFTISTVQAEDLAVYFCQQDYSSPWTFGGGTKLEIK

SEQ ID NO: 88 - protein, 8 aa, synthetic construct
  REGION 1..8: note = CDR1 VH_9A2.7
GYNFTTFW

SEQ ID NO: 89 - protein, 8 aa, synthetic construct
  REGION 1..8: note = CDR2 VH_9A2.7
IYPSDSYA

SEQ ID NO: 90 - protein, 13 aa, synthetic construct
  REGION 1..13: note = CDR3 VH_9A2.7
TRPSYFGRNSFAY

SEQ ID NO: 91 - protein, 120 aa, synthetic construct
  REGION 1..120: note = VH_9A2.7
QVQLQQPGAELVRPGASVKLSCKASGYNFTTFWINWVKQRPGQGLEWIGNIYPSDSYANYNQKFKDKATLTVDKSSTTAYMQLSSPTSEDSAVYYCTRPSYFGRNSFAYWGQGTLVTVSA

SEQ ID NO: 92 - protein, 12 aa, synthetic construct
  REGION 1..12: note = CDR1 VK_9A2.7
QSLLYSVNHKNY

SEQ ID NO: 93 - skipped

SEQ ID NO: 94 - protein, 9 aa, synthetic construct
  REGION 1..9: note = CDR3 VK_9A2.7
HQYYTYPLT

SEQ ID NO: 95 - protein, 113 aa, synthetic construct
  REGION 1..113: note = VK_9A2.7
DIVMTQSPSSLVVSVGEKVTMSCKSSQSLLYSVNHKNYLAWYQQKPGQSPKLLIYWASTRESGVPDRFTGSGSGTDFSLTISSVKAEDLAVYYCHQYYTYPLTFGAGTKLELK

SEQ ID NO: 96 - protein, 8 aa, synthetic construct
  REGION 1..8: note = CDR1 VH_3A1.4
GDSITSGY

SEQ ID NO: 97 - protein, 7 aa, synthetic construct
  REGION 1..7: note = CDR2 VH_3A1.4
ISNSGIT

SEQ ID NO: 98 - protein, 15 aa, synthetic construct
  REGION 1..15: note = CDR3 VH_3A1.4
TRFGSTMILYYTMDY

SEQ ID NO: 99 - protein, 121 aa, synthetic construct
  REGION 1..121: note = VH_3A1.4
DVQLQESGPSLVKPSQTLSLTCSVTGDSITSGYWNWIRKFPGNKLEYMGYISNSGITYYNPSLKSRISITRDTSKNQYFLQLNSVTAEDTATYYCTRFGSTMILYYTMDYWGQGTSVTVSS

SEQ ID NO: 100 - protein, 6 aa, synthetic construct
  REGION 1..6: note = CDR1 VK_3A1.4
QSISDY

SEQ ID NO: 101 - skipped

SEQ ID NO: 102 - protein, 9 aa, synthetic construct
  REGION 1..9: note = CDR3 VK_3A1.4
QNGHSFPLT

SEQ ID NO: 103 - protein, 107 aa, synthetic construct
  REGION 1..107: note = VK_3A1.4
DIVMTQSPVTLSVTPGDRVSLSCRASQSISDYLHWYQQKSQESPRLLIKYASKSISGIPSRFSGSGSGSNFTLSINSVEPEDVGVYYCQNGHSFPLTFGAGTKLELK

SEQ ID NO: 104 - protein, 8 aa, synthetic construct
  REGION 1..8: note = CDR1 VH_8F06
GYTFTSYV

SEQ ID NO: 105 - protein, 8 aa, synthetic construct
  REGION 1..8: note = CDR2 VH_8F06
INPYNDGT

SEQ ID NO: 106 - protein, 6 aa, synthetic construct
  REGION 1..6: note = CDR3 VH_8F06
VTLFAY

SEQ ID NO: 107 - protein, 113 aa, synthetic construct
  REGION 1..113: note = VH_8F06
EVQLQQSGPELVKPGASVKMSCKASGYTFTSYVMHWVKQKPGQGLEWIGYINPYNDGTKYNEKFKGKATLTSDKSSSTAYMELSSLTSEDSAVYYCVTLFAYWGQGTLVTVSA

SEQ ID NO: 108 - protein, 5 aa, synthetic construct
  REGION 1..5: note = CDR1 VK_8F06
SSISY

SEQ ID NO: 109 - skipped

SEQ ID NO: 110 - protein, 9 aa, synthetic construct
  REGION 1..9: note = CDR3 VK_8F06
HQRSSYPFT

SEQ ID NO: 111 - protein, 106 aa, synthetic construct
  REGION 1..106: note = VK_8F06
QIVLTQSPAIMSASPGEKVTMTCSASSSISYMHWYQQKPGTSPKRWIYDTSKLASGVPARFSGSGSGTSYSLTISSMEAEDAATYYCHQRSSYPFTFGSGTKLEIK

SEQ ID NO: 112 - protein, 4 aa, synthetic construct
GAGG

SEQ ID NO: 113 - protein, 4 aa, synthetic construct
GGAG

SEQ ID NO: 114 - protein, 4 aa, synthetic construct
GVGG

SEQ ID NO: 115 - protein, 4 aa, synthetic construct
GGVG

SEQ ID NO: 116 - protein, 4 aa, synthetic construct
GGFG

SEQ ID NO: 117 - protein, 4 aa, synthetic construct
GFGG

SEQ ID NO: 118 - protein, 4 aa, synthetic construct
GGSG

SEQ ID NO: 119 - protein, 5 aa, synthetic construct
GGSGG

SEQ ID NO: 120 - protein, 5 aa, synthetic construct
GSGSG

SEQ ID NO: 121 - protein, 5 aa, synthetic construct
GSGGG

SEQ ID NO: 122 - protein, 5 aa, synthetic construct
GGGSG

SEQ ID NO: 123 - protein, 5 aa, synthetic construct
GSSSG

SEQ ID NO: 124 - protein, 5 aa, synthetic construct
GSGGS

SEQ ID NO: 125 - protein, 4 aa, synthetic construct
GGGS